European Patent Specification EP 4 029 952 B1, published January 1, 2025. Title: ENZYME- AND AMPLIFICATION-FREE SEQUENCING. Applicant: NanoString Technologies, Inc. Application Divisional of EP20151469.2. The sequence listing filed with the application follows.

SEQUENCE LISTING (104 sequences)

SEQ ID NO: 1 - DNA, 10 bp, Artificial Sequence
  Synthetic Polynucleotide
atacatctag

SEQ ID NO: 2 - DNA, 10 bp, Artificial Sequence
  Synthetic Polynucleotide
gatctacata

SEQ ID NO: 3 - DNA, 10 bp, Artificial Sequence
  Synthetic Polynucleotide
ttaggtaaag

SEQ ID NO: 4 - DNA, 10 bp, Artificial Sequence
  Synthetic Polynucleotide
tcttcattac

SEQ ID NO: 5 - DNA, 10 bp, Artificial Sequence
  Synthetic Polynucleotide
atgaatctac

SEQ ID NO: 6 - DNA, 10 bp, Artificial Sequence
  Synthetic Polynucleotide
tcaatgtatg

SEQ ID NO: 7 - DNA, 10 bp, Artificial Sequence
  Synthetic Polynucleotide
aattgagtac

SEQ ID NO: 8 - DNA, 10 bp, Artificial Sequence
  Synthetic Polynucleotide
atgttaatgg

SEQ ID NO: 9 - DNA, 10 bp, Artificial Sequence
  Synthetic Polynucleotide
aattaggatg

SEQ ID NO: 10 - DNA, 10 bp, Artificial Sequence
  Synthetic Polynucleotide
ataatggatc

SEQ ID NO: 11 - DNA, 10 bp, Artificial Sequence
  Synthetic Polynucleotide
taataaggtg

SEQ ID NO: 12 - DNA, 10 bp, Artificial Sequence
  Synthetic Polynucleotide
tagttagagc

SEQ ID NO: 13 - DNA, 10 bp, Artificial Sequence
  Synthetic Polynucleotide
atagagaagg

SEQ ID NO: 14 - DNA, 10 bp, Artificial Sequence
  Synthetic Polynucleotide
ttgatgatac

SEQ ID NO: 15 - DNA, 10 bp, Artificial Sequence
  Synthetic Polynucleotide
atagtgattc

SEQ ID NO: 16 - DNA, 10 bp, Artificial Sequence
  Synthetic Polynucleotide
tataacgatg

SEQ ID NO: 17 - DNA, 10 bp, Artificial Sequence
  Synthetic Polynucleotide
ttaagtttag

SEQ ID NO: 18 - DNA, 10 bp, Artificial Sequence
  Synthetic Polynucleotide
atacgttatg

SEQ ID NO: 19 - DNA, 10 bp, Artificial Sequence
  Synthetic Polynucleotide
tgtactatag

SEQ ID NO: 20 - DNA, 10 bp, Artificial Sequence
  Synthetic Polynucleotide
ttaacaagtg

SEQ ID NO: 21 - DNA, 10 bp, Artificial Sequence
  Synthetic Polynucleotide
aactatgtac

SEQ ID NO: 22 - DNA, 10 bp, Artificial Sequence
  Synthetic Polynucleotide
taactatgac

SEQ ID NO: 23 - DNA, 10 bp, Artificial Sequence
  Synthetic Polynucleotide
actaatgttc

SEQ ID NO: 24 - DNA, 10 bp, Artificial Sequence
  Synthetic Polynucleotide
tcattgaatg

SEQ ID NO: 25 - DNA, 14 bp, Artificial Sequence
  Synthetic Polynucleotide
ctgtctcatctctt

SEQ ID NO: 26 - DNA, 26 bp, Artificial Sequence
  Synthetic Polynucleotide
ctgtctcatctcttgctgcatcctgt

SEQ ID NO: 27 - DNA, 38 bp, Artificial Sequence
  Synthetic Polynucleotide
ctgtctcatctcttgctgcatcctgtcggttcacgttg

SEQ ID NO: 28 - DNA, 36 bp, Artificial Sequence
  Synthetic Polynucleotide
ctgtctcatcttgctgcatcctgtcggttcacgttg

SEQ ID NO: 29 - DNA, 36 bp, Artificial Sequence
  Synthetic Polynucleotide
ctgtctcattttgctgcatcctgtccgttcacgttg

SEQ ID NO: 30 - DNA, 43 bp, Artificial Sequence
  Synthetic Polynucleotide
gactgtacccacgcgatgacgttcgtcaagagtcgcataatct

SEQ ID NO: 31 - DNA, 44 bp, Artificial Sequence
  Synthetic Polynucleotide
agactgtaccacaagaatccctgctagctgaaggagggtcaaac

SEQ ID NO: 32 - DNA, 45 bp, Artificial Sequence
  Synthetic Polynucleotide
gagactgtaccctacgtatatatccaagtggttatgtccgacggc

SEQ ID NO: 33 - DNA, 46 bp, Artificial Sequence
  Synthetic Polynucleotide
tgagactgtaccacccctccaaacgcattcttattggcaaatggaa

SEQ ID NO: 34 - DNA, 47 bp, Artificial Sequence
  Synthetic Polynucleotide
ctgagactgtacccgggaatcggcatttcgcattcttaggatctaaa

SEQ ID NO: 35 - DNA, 44 bp, Artificial Sequence
  Synthetic Polynucleotide
caatgtgagtctcttggtacagtctcagttagtcactccctaag

SEQ ID NO: 36 - DNA, 45 bp, Artificial Sequence
  Synthetic Polynucleotide
gagacagtaccctggtctaggtatctaattcgtgggtcgggtact

SEQ ID NO: 37 - DNA, 45 bp, Artificial Sequence
  Synthetic Polynucleotide
gagaccgtaccgctcattttgaacatacgattgcgattacggaaa

SEQ ID NO: 38 - DNA, 45 bp, Artificial Sequence
  Synthetic Polynucleotide
gagacggtaccttaaagctatccacgaatgtcaaaaatgtggttt

SEQ ID NO: 39 - DNA, 45 bp, Artificial Sequence
  Synthetic Polynucleotide
gagagtgtacccaatgcttgcagtatgtatcctgatcgtgcgtgc

SEQ ID NO: 40 - DNA, 45 bp, Artificial Sequence
  Synthetic Polynucleotide
gagaatgtaccctcataccaatgtaaagtatagttaacgccctgt

SEQ ID NO: 41 - DNA, 45 bp, Artificial Sequence
  Synthetic Polynucleotide
gagattgtaccctacatatataggaaaagggaaggtagaagagct

SEQ ID NO: 42 - DNA, 12 bp, Artificial Sequence
  Synthetic Polynucleotide
cacgaacgtcag

SEQ ID NO: 43 - DNA, 12 bp, Artificial Sequence
  Synthetic Polynucleotide
catcgcatgcct

SEQ ID NO: 44 - DNA, 12 bp, Artificial Sequence
  Synthetic Polynucleotide
gtcatctcctac

SEQ ID NO: 45 - DNA, 12 bp, Artificial Sequence
  Synthetic Polynucleotide
gtcatccgctac

SEQ ID NO: 46 - DNA, 12 bp, Artificial Sequence
  Synthetic Polynucleotide
gtcatcgactac

SEQ ID NO: 47 - DNA, 12 bp, Artificial Sequence
  Synthetic Polynucleotide
gtcatcttctac

SEQ ID NO: 48 - DNA, 12 bp, Artificial Sequence
  Synthetic Polynucleotide
gtcatcacctac

SEQ ID NO: 49 - DNA, 12 bp, Artificial Sequence
  Synthetic Polynucleotide
gtcatcactcac

SEQ ID NO: 50 - DNA, 12 bp, Artificial Sequence
  Synthetic Polynucleotide
gtcatcttcgac

SEQ ID NO: 51 - DNA, 12 bp, Artificial Sequence
  Synthetic Polynucleotide
gtcatcaactac

SEQ ID NO: 52 - DNA, 12 bp, Artificial Sequence
  Synthetic Polynucleotide
gtcatccgtaac

SEQ ID NO: 53 - DNA, 12 bp, Artificial Sequence
  Synthetic Polynucleotide
gtcatccgaaac

SEQ ID NO: 54 - DNA, 12 bp, Artificial Sequence
  Synthetic Polynucleotide
gtcatcacaaac

SEQ ID NO: 55 - DNA, 12 bp, Artificial Sequence
  Synthetic Polynucleotide
gtcatcttgcac

SEQ ID NO: 56 - DNA, 12 bp, Artificial Sequence
  Synthetic Polynucleotide
gtcatcttgcct

SEQ ID NO: 57 - DNA, 12 bp, Artificial Sequence
  Synthetic Polynucleotide
gtcatccgtcct

SEQ ID NO: 58 - DNA, 12 bp, Artificial Sequence
  Synthetic Polynucleotide
cttttcacctct

SEQ ID NO: 59 - DNA, 12 bp, Artificial Sequence
  Synthetic Polynucleotide
cttttcctctct

SEQ ID NO: 60 - DNA, 12 bp, Artificial Sequence
  Synthetic Polynucleotide
cttttcgactct

SEQ ID NO: 61 - DNA, 12 bp, Artificial Sequence
  Synthetic Polynucleotide
cttttctgctct

SEQ ID NO: 62 - DNA, 12 bp, Artificial Sequence
  Synthetic Polynucleotide
cttttctgtact

SEQ ID NO: 63 - DNA, 12 bp, Artificial Sequence
  Synthetic Polynucleotide
cttttctgtgct

SEQ ID NO: 64 - DNA, 12 bp, Artificial Sequence
  Synthetic Polynucleotide
cttttctgtcct

SEQ ID NO: 65 - DNA, 12 bp, Artificial Sequence
  Synthetic Polynucleotide
cttttcactcct

SEQ ID NO: 66 - DNA, 12 bp, Artificial Sequence
  Synthetic Polynucleotide
cttttcgttcct

SEQ ID NO: 67 - DNA, 12 bp, Artificial Sequence
  Synthetic Polynucleotide
cttttcgtacct

SEQ ID NO: 68 - DNA, 12 bp, Artificial Sequence
  Synthetic Polynucleotide
cttttccgtcct

SEQ ID NO: 69 - DNA, 12 bp, Artificial Sequence
  Synthetic Polynucleotide
cttttctgacct

SEQ ID NO: 70 - DNA, 12 bp, Artificial Sequence
  Synthetic Polynucleotide
aggcatgcgatg

SEQ ID NO: 71 - DNA, 12 bp, Artificial Sequence
  Synthetic Polynucleotide
aggcattgtgct

SEQ ID NO: 72 - DNA, 12 bp, Artificial Sequence
  Synthetic Polynucleotide
aggcattgctct

SEQ ID NO: 73 - DNA, 12 bp, Artificial Sequence
  Synthetic Polynucleotide
aggcatttctac

SEQ ID NO: 74 - DNA, 12 bp, Artificial Sequence
  Synthetic Polynucleotide
aggcatacctac

SEQ ID NO: 75 - DNA, 12 bp, Artificial Sequence
  Synthetic Polynucleotide
aggcatttgcac

SEQ ID NO: 76 - DNA, 12 bp, Artificial Sequence
  Synthetic Polynucleotide
aggcatcgtcct

SEQ ID NO: 77 - DNA, 12 bp, Artificial Sequence
  Synthetic Polynucleotide
tcctgtcggttc

SEQ ID NO: 78 - DNA, 12 bp, Artificial Sequence
  Synthetic Polynucleotide
gttcaatgctct

SEQ ID NO: 79 - DNA, 12 bp, Artificial Sequence
  Synthetic Polynucleotide
attcggtgctct

SEQ ID NO: 80 - DNA, 12 bp, Artificial Sequence
  Synthetic Polynucleotide
gatgcctgctct

SEQ ID NO: 81 - DNA, 12 bp, Artificial Sequence
  Synthetic Polynucleotide
tttgcttgctct

SEQ ID NO: 82 - DNA, 100 bp, Artificial Sequence
  Synthetic Polynucleotide
ttcactgtagctgtctcattttgctgcatcctgtccgttcacgttggagcttgtcatccgtcctcttttcactcctaggcatttgcctattcggcgtcct

SEQ ID NO: 83 - DNA, 10 bp, Artificial Sequence
  Synthetic Polynucleotide
cgatctggtt

SEQ ID NO: 84 - DNA, 10 bp, Artificial Sequence
  Synthetic Polynucleotide
cgatctggtt

SEQ ID NO: 85 - DNA, 10 bp, Artificial Sequence
  Synthetic Polynucleotide
gctagaccaa

SEQ ID NO: 86 - DNA, 10 bp, Artificial Sequence
  Synthetic Polynucleotide
gctggaccaa

SEQ ID NO: 87 - DNA, 10 bp, Artificial Sequence
  Synthetic Polynucleotide
gctcgaccaa

SEQ ID NO: 88 - DNA, 10 bp, Artificial Sequence
  Synthetic Polynucleotide
gcttgaccaa

SEQ ID NO: 89 - DNA, 10 bp, Artificial Sequence
  Synthetic Polynucleotide
gagactgtac

SEQ ID NO: 90 - DNA, 10 bp, Artificial Sequence
  Synthetic Polynucleotide
gagacagtac

SEQ ID NO: 91 - DNA, 10 bp, Artificial Sequence
  Synthetic Polynucleotide
gagaccgtac

SEQ ID NO: 92 - DNA, 10 bp, Artificial Sequence
  Synthetic Polynucleotide
gagacggtac

SEQ ID NO: 93 - DNA, 10 bp, Artificial Sequence
  Synthetic Polynucleotide
gagagtgtac

SEQ ID NO: 94 - DNA, 10 bp, Artificial Sequence
  Synthetic Polynucleotide
gagaatgtac

SEQ ID NO: 95 - DNA, 10 bp, Artificial Sequence
  Synthetic Polynucleotide
gagattgtac

SEQ ID NO: 96 - DNA, 10 bp, Artificial Sequence
  Synthetic Polynucleotide
gagactgtac

SEQ ID NO: 97 - DNA, 10 bp, Artificial Sequence
  Synthetic Polynucleotide
gagattgtac

SEQ ID NO: 98 - DNA, 10 bp, Artificial Sequence
  Synthetic Polynucleotide
gagaccgtac

SEQ ID NO: 99 - DNA, 10 bp, Artificial Sequence
  Synthetic Polynucleotide
gagagtgtac

SEQ ID NO: 100 - DNA, 12 bp, Artificial Sequence
  Synthetic Polynucleotide
ctgagactgtac

SEQ ID NO: 101 - DNA, 11 bp, Artificial Sequence
  Synthetic Polynucleotide
tgagactgtac

SEQ ID NO: 102 - DNA, 10 bp, Artificial Sequence
  Synthetic Polynucleotide
gagactgtac

SEQ ID NO: 103 - DNA, 12 bp, Artificial Sequence
  Synthetic Polynucleotide
catgtcagagtc

SEQ ID NO: 104 - DNA, 11 bp, Artificial Sequence
  Synthetic Polynucleotide
catgtcagagt